European Patent Application EP 4 253 551 A2, published October 4, 2023. Title: NOVEL CRISPR DNA AND RNA TARGETING ENZYMES AND SYSTEMS. Applicant: ARBOR BIOTECHNOLOGIES, INC. Application EP. The sequence listing filed with the application follows.

SEQUENCE LISTING (493 sequences)

SEQ ID NO: 1 - protein, 772 aa, unidentified
  REGION 1..772: note = source = /note="Description of Unknown: bioreactor-anaerobic-anaerobic digester digestate sequence"
MTRIKYRQERTLVRGLQRLPNQDKAEFNKNVLGLRRHFEQFNLNVAELCQWLISFKPENPGSVCETKLFWEFMLEPENFCPDTYDRGPDWLRHEIFVLAAGWRTFEDIKAHNMPESLFESIKIASSKPRSKTAEALFIRLKSLEASHVMVLLKSASEWLSTRYVRQSENWKQNEQEWQKKKAAWEDKHPELTPAIRDKYNAIFVELGISEKRPHVCSWKKLSENKDNCDWAGERKNIGDKWISHSDLCIKYHEFARKLRSKQRQHFVDNANQYLELRRRYPQWTRDMAMNGLFKNVPLARNWFRNAWTNYLNALNILETTILENYSGHLPHCEKLSDECVFKKHTDNCRRYKLLLGEKLSNQERELEETYREWRREFLAPPNKPFLRYPSAQKLPTPKLFGRGYYDLDFTRHVVKLRLDDMPADNFVSFGFKPWPRGYDKKPGEINITSVHVHFIGTRARVGFRFAVPHSDSRFSVSQDKIDELRSGGFPGKSQDQEFLNEARQRLLDGMNENQKSALRIMAVDLGTHRAAAAFFTGCIFNKAKLLKLKKIDLLTEPKTDTTKPEKLSADEKKIQREKGLTQHHVGKHFETLEARTKEIISKRQNMKMAPSDDTPDIVGDHDLRHLTSHIRRMIRDWVRLNARQITELAEEENVDLIVFESMRGFRAPGYDKLDLKKKRRLAFFAYGQIRRKVAEKAVERGMRVITVPYFKSSQICAQCGRSQNDKNKLRDNKWKQSFQCEFSDCNYKTHSDENAARVLGRVFWGEITLPTD

SEQ ID NO: 2 - protein, 821 aa, unidentified
  REGION 1..821: note = source = /note="Description of Unknown: activated sludge metagenome sequence"
MLPTRYKPARTLVRPLGRLPHEPRKEFVEKCRRVRMHFEQFNIDVADLCQWLMSLRPNTRIGDAQSTVFWDFFLNPSILTVEADEKERDRWRLAAFDELLQIRFGHDPNAPPWSEEFRSAIRHVAQRPKSATAQRLFDRLRSLTAPHRLVLLKSAAEWIIARYQRGMENWQRQFAEWQREKEEWEAAHPNLTPEVRDAFTRVFKNLFENPDGDGKIGVRRKNPRICSWERLKLNKDNCVYAGQKGHGPLCWEFSKFVKAQKNAGTIKTFFVDVANKYLHVRRNLSKPGVKLKKSPRQEAFKRLYNQKGMEKARNWFTDAWSGYLTALNLNEKTILDHGCLKHCGAIGAEFEKSLCQFNPHTHLCVQYRNALESLEPAIRELEGDYREWRRLFLAPPRKPSFRYPSSRRLPMPKIFGEHFHQIDFDQSILRLRLEDMAEGEWIEFGFKPWPKDYRPGKDEVRVTSVHVNFHGNRMRAGFHFEAPAKPSRFACTQDELDDLRSKQFPRQSQDRQLLEVARRRLLESFDGMLESDLRILAVDLGEKGAAAAVYQGHGHEADVAIPIVKIDRLYDHVPDVLDVESARVPPPKFDDSRDPRGVRKEHVGRHLGQLQRGAQTLAQHRQQDESAPAALRRHDFRSLTRHIRWMIRDWTRHNAAQITAAAETHRCHLIVFESLRGFKPRGYDQMDFAQKARLAFFAYGRVRRKVVEKAVERGLRVVTVPYGFTSQICSECGHRQRNKGRLRKNKYQRRFVCECGEPKKSANKTAAPDRSATVSPCTCRLQLGSDVNAARVLARVFWDEIVLPTREEMREPAVDSAPPSK

SEQ ID NO: 3 - protein, 786 aa, unidentified
  REGION 1..786: note = source = /note="Description of Unknown: activated sludge metagenome sequence"
MHFEQFNIDVADLCQWLMSLRPNTRIGDAQSTVFWDFFLNPSILTVEADEKERDRWRLAAFDELLQIRFGHDPNAPPWSEEFRSAIRHVAQRPKSATAQRLFDRLRSLTAPHRLVLLKSAAEWIIARYQRGMENWQRQFAEWQREKEEWEAAHPNLTPEVRDAFTRVFKNLFENPDGDGKIGVRRKNPRICSWERLKLNKDNCVYAGQKGHGPLCWEFSKFVKAQKNAGTIKTFFVDVANKYLHVRRNLSKPGVKLKKSPRQEAFKRLYNQKGMEKARNWFTDAWSGYLTALNLNEKTILDHGCLKHCGAIGAEFEKSLCQFNPHTHLCVQYRNALESLEPAIRELEGDYREWRRLFLAPPRKPSFRYPSSRRLPMPKIFGEHFHQIDFDQSILRLRLEDMAEGEWIEFGFKPWPKDYRPGKDEVRVTSVHVNFHGNRMRAGFHFEAPAKPSRFACTQDELDDLRSKQFPRQSQDRQLLEVARRRLLESFDGMLESDLRILAVDLGEKGAAAAVYQGHGHEADVAIPIVKIDRLYDHVPDVLDVESARVPPPKFDDSRDPRGVRKEHVGRHLGQLQRGAQTLAQHRQQDESAPAALRRHDFRSLTRHIRWMIRDWTRHNAAQITAAAETHRCHLIVFESLRGFKPRGYDQMDFAQKARLAFFAYGRVRRKVVEKAVERGLRVVTVPYGFTSQICSECGHRQRNKGRLRKNKYQRRFVCECGEPKKSANKTAAPDRSATVSPCTCRLQLGSDVNAARVLARVFWDEIVLPTREEMREPAVDSAPPSK

SEQ ID NO: 4 - protein, 769 aa, unidentified
  REGION 1..769: note = source = /note="Description of Unknown: candidate division Zixibacteria bacterium Bacteria. sequence"
MNRTRYREERTITRGMRRLPGEERKSFKAKVITLRRNFEQFNTDVSEICQWLMSIRPNGKHNIPNTEPFWDFILEPHNFVVNQEETNIDSVRLVVFEMAVGWRQVTDVANFELERQLLMSLESIQSVPRTIAAKRMLQRIKNYEFQHKMVLLRSAVEWINTRFIRTYKNWEMNIKEFLEKKKVWENDHPKLTEEIRNTFNKVFDELEISKKNPNICRWSHLKKNRDNCNYAGVRIKVGGEYNNHSEKCKRYQDFLKKHSAHKKYFAANAMMYINIRKKRRDLTKREAIKVLLDKIPQARSWFPQAWDNYLEYLGLNEISLINKFDGQLPHCLRLDTECIYNVHTQSCRKYYVLLKDLPDKYLSLEETYREWRKYFLREPRKPVFAYPSTRQRTVSKIFGRDYFEADYDNSIIKLRLDDMAEGQFLSFGFKPWPVDYDVQPIDTEITSVLVHFIGTRARVGFRFKMPHRPSRINIKQDELDELRSRSRLIQEKDQALLEKVRLRLRDGFIGIFDKELRVLAVDLGTSSCATAFFVGRQFQESSRLQIVKYDRVYKSNYEIKKRRNNKGIDKQKQLLFKEKGLNQYHIKVHLDKLAEQNKQIIKKREASGNPTPTEQDMRRLSLHIGWMHRDWVRINASQIIKSAKKLRADLIVFESLRDFRPMMFNEFDIDKKRRLAFFPFGLIRHKVIEKAVESGMRVVTVPYMFSSQFCGACGRQQNDKKRLQKNKTDKRGACFICEYNDCAFEGDPDENAARVLGGVFWGNIGLPLS

SEQ ID NO: 5 - protein, 830 aa, unidentified
  REGION 1..830: note = source = /note="Description of Unknown: aquatic-thermal springs-hot spring sediment sequence"
MHPSRYKTARTLVRRLCRLPGEDRSAFRSKVGLLRGHFEQFNVDVSELCQWLMSLRKRNKVPENPATFGALGDFLLQPGLPGEETDEKEADRLRLAVFDAVAGFRMLEDRLAASIPASLSDAIRDEAVFLAGVRAAGKPSGLARVLARLEACAPAQRLVLLKSAAEWIVARFLRGTENWMRQRAEWEKEKAAWEAAHPHLTPEVRAQFNKIFESLHDPENSGKPGVSRKNPRICPWDRLKQNLDNCCYGEKGHSALCWRYQDFLKQRMGENRRDKKNFSATAMDLAQICREWKIQHSRNALNNPRVLDRLFAEHERRKQDKTKKESRSPKPRQGGYKANPKADYLRSFKAHWKAYLEHMKLNDTTVLERGCLPHCLSIKKNGKESTCKWNKHTELCLEYKRSLAPLPDSVLELEPEYREWRRLYLHGPGRPHFRYPSAGELPLPKVFGEGFHQVDLDRSIVRLRLEGAAEGEWLEFGFIPWPRGYQPSRREVLITSVQVHFVGTRPRAGFRFDVSHRTSRFGCSQDELDELRSRRYPRQAQDKEFLAAARAQLIQTFEGGEGAARQQMRVMSVDLGEGGACASIYEGRTHQKDESLKVIKIDRRYDQHPEVLEKDVGAAKPQKFEKSDPRGVRKEHVARHLNRIAAGASAIAEHRRKERSDAECSVGELQEHDFRSLKRHIAWMIRDWVRLNAAQIIDVAKQHCCDLIVFESQRGFRLPGYDELDRGKKQRFAILAFGRIRRKVVEKAVEHGMRVVTVPYFASSQVCSACKRVQENRGSWRENKKKRVFACEFCKLKLNSDANASRVLARVFWGEIELPEPTRAHLPSKA

SEQ ID NO: 6 - protein, 767 aa, unidentified
  REGION 1..767: note = source = /note="Description of Unknown: aquatic-thermal springs-hot spring sediment sequence"
MAQASSTPAVSPRPRPRYREERTLVRKLLPRPGQSKQEFRENVKKLRKAFLQFNADVSGVCQWAIQFRPRYGKPAEPTETFWKFFLEPETSLPPNDSRSPEFRRLQAFEAAAGINGAAALDDPAFTNELRDSILAVASRPKTKEAQRLFSRLKDYQPAHRMILAKVAAEWIESRYRRAHQNWERNYEEWKKEKQEWEQNHPELTPEIREAFNQIFQQLEVKEKRVRICPAARLLQNKDNCQYAGKNKHSVLCNQFNEFKKNHLQGKAIKFFYKDAEKYLRCGLQSLKPNVQGPFREDWNKYLRYMNLKEETLRGKNGGRLPHCKNLGQECEFNPHTALCKQYQQQLSSRPDLVQHDELYRKWRREYWREPRKPVFRYPSVKRHSIAKIFGENYFQADFKNSVVGLRLDSMPAGQYLEFAFAPWPRNYRPQPGETEISSVHLHFVGTRPRIGFRFRVPHKRSRFDCTQEELDELRSRTFPRKAQDQKFLEAARKRLLETFPGNAEQELRLLAVDLGTDSARAAFFIGKTFQQAFPLKIVKIEKLYEQWPNQKQAGDRRDASSKQPRPGLSRDHVGRHLQKMRAQASEIAQKRQELTGTPAPETTTDQAAKKATLQPFDLRGLTVHTARMIRDWARLNARQIIQLAEENQVDLIVLESLRGFRPPGYENLDQEKKRRVAFFAHGRIRRKVTEKAVERGMRVVTVPYLASSKVCAECRKKQKDNKQWEKNKKRGLFKCEGCGSQAQVDENAARVLGRVFWGEIELPTAIP

SEQ ID NO: 7 - protein, 720 aa, unidentified
  REGION 1..720: note = source = /note="Description of Unknown: aquatic-sediment-hot spring sediment sequence"
MSIRPDAKKPDKETKSFWDFFLNPESFFDPTINNVDIIRLNLFKVITGRESEANLIRYNLPLLLYESIILLKKQEPSDTARRLFARLKKMEPVHVMILLKAAAEWVYARYQRLMDNHEYQYKVWHDEKSAWENKHPELTPEIREKYNSIFKELGRKQGVTIRKNPRICNWEKLEENKDNCGYNGKRIQFGDKWKAHSMLCIEYRNFLRDNKITGKRIGFFATHAYNYLKLRAHQPRLTKDEAFKRIFKSAPNGIYWFPKAWKNYLQFMNLNELNLIRKYNANLPHCLEFKGDKDCQYNKHTELCQEYKTLLLEKFTEDELKLEGLYREWRKQYLSGPSKPAFRYPSCSKLPTPKIFGKRFHEIDFENSIVRLRLDDMPDGEYLTFKFKPWPNDYQPQPEEAEISSVHVHFVGTRARVGFRFKIAHKQSRFKTSQDEIDELRSRKYPRQAQDADFLKAAREKLLQSFKGENPTKEIKIMAVDLGEYRGYISVYKGENIEISEPLSILKIDKLYDSLESAGVDKTDLAKYIKDHKGLIKEHVDSHLKVISEKANEITKHRPAGKKTGASNLKDYDLRSLTAHTGWMIRDWVRLNVSQIIRIAEKHEVDLIVLESLRGWKAPGYDEFDLRKKRWLAFFSYGRIRHKLKEKAVERGMMVVTVPYYKSSQICSKCGKEQENKGLWKKNKNERLFICDYPGCGHRDNSDANAAKVLAKIFWGEIVL

SEQ ID NO: 8 - protein, 774 aa, unidentified
  REGION 1..774: note = source = /note="Description of Unknown: aquatic-sediment-hot spring sediment sequence"
MDNNRTRYREERTLVRSLRPLDGENRNAFKNRVNRLRIHFKNFNLDVSEICQWLMSIRPDAKKPDKETKSFWDFFLNPESFFDPTINNVDIIRLNLFKVITGRESEANLIRYNLPLLLYESIILLKKQEPSDTARRLFARLKKMEPVHVMILLKAAAEWVYARYQRLMDNHEYQYKVWHDEKSAWENKHPELTPEIREKYNSIFKELGRKQGVTIRKNPRICNWEKLEENKDNCGYNGKRIQFGDKWKAHSMLCIEYRNFLRDNKITGKRIGFFATHAYNYLKLRAHQPRLTKDEAFKRIFKSAPNGIYWFPKAWKNYLQFMNLNELNLIRKYNANLPHCLEFKGDKDCQYNKHTELCQEYKTLLLEKFTEDELKLEGLYREWRKQYLSGPSKPAFRYPSCSKLPTPKIFGKRFHEIDFENSIVRLRLDDMPDGEYLTFKFKPWPNDYQPQPEEAEISSVHVHFVGTRARVGFRFKIAHKQSRFKTSQDEIDELRSRKYPRQAQDADFLKAAREKLLQSFKGENPTKEIKIMAVDLGEYRGYISVYKGENIEISEPLSILKIDKLYDSLESAGVDKTDLAKYIKDHKGLIKEHVDSHLKVISEKANEITKHRPAGKKTGASNLKDYDLRSLTAHTGWMIRDWVRLNVSQIIRIAEKHEVDLIVLESLRGWKAPGYDEFDLRKKRWLAFFSYGRIRHKLKEKAVERGMMVVTVPYYKSSQICSKCGKEQENKGLWKKNKNERLFICDYPGCGHRDNSDANAAKVLAKIFWGEIVL

SEQ ID NO: 9 - DNA, 36 bp, synthetic construct
  misc_feature 1..36: note = source = /note="Description of Artificial Sequence: Synthetic oligonucleotide"
  source 1..36: mol_type = other DNA
gttgtagcggcccctgaattagcggtttccgacacc

SEQ ID NO: 10 - DNA, 36 bp, synthetic construct
  misc_feature 1..36: note = source = /note="Description of Artificial Sequence: Synthetic oligonucleotide"
  source 1..36: mol_type = other DNA
ggtgcggcagccggtagaactgcggcttccgacacc

SEQ ID NO: 11 - DNA, 36 bp, synthetic construct
  misc_feature 1..36: note = source = /note="Description of Artificial Sequence: Synthetic oligonucleotide"
  source 1..36: mol_type = other DNA
gttggagtcagcaaggaatcaacggttttggacacc

SEQ ID NO: 12 - skipped

SEQ ID NO: 13 - DNA, 36 bp, synthetic construct
  misc_feature 1..36: note = source = /note="Description of Artificial Sequence: Synthetic oligonucleotide"
  source 1..36: mol_type = other DNA
ggtggaaagggccggagatttaccggctctgacacc

SEQ ID NO: 14 - skipped

SEQ ID NO: 15 - protein, 761 aa, Planctomycetes bacterium
MGLRKRYVELCDNSGLRADLSSFGTLGNFLLEPSLDGSEADERERDRWRLAVFDIVAGFRADIQLDGRTLPNELRQAITDAADQMRNTIADGKKKTGLRRLFQRLGDLEEAHRLVLLKSAAEWIVARYLRSVENWVRQHTEWEKEKQQWESHKDNKTDHTLLTPDIREKYTAVFKLLVWDKDKPPGVRNKRPRICPYDRLKQNIDNCCYAGQKGHGPLCWKYNEFVKARKARNPSFNDKKFAEDVAKYLPPRAKGEQRHLILKAIFPNKQQDQQRFSDNWTAYLSAMKLNEQTLVQHQQLPHCLKIGETFEKSACVWNPHTDLCGQYHRALVNPNNGFDDAMLSLEPLYRAWRRNYLAGPRKPSFRYPASRDLPMPKIFGDGFHEVDFENSIVRLRLDDMPRGQWLDLGFTPWPRGYKPSRAEISEPGRVTSVHVHFVGVRARIGFRFEVAHAPSRFGCTQDEIDELRSRHYPRQAQDQEFLEAARKCLLDSMTEGSENDLRIMAVDLGEKGACAAVYRGRTREMDIPLAIVKINKLYEKPPKTLEPDRHSRPEESKRKFEEADPRGVRKEHVGRHLERVAAMSQEIAKHRQPAVATTVTVSVNDLRGLKRHVAWMIRDWARHNASQIVKAAEEHQCDVIVFESLRGFRPPGYDKLDEMSAKKKRWLAMFAYGRVRRKVIEKAVERGMRVVTVPYFKSSQVCSDCGREQVNVGLLRKNKLSKGQFVCENCKVTLTSDANAARVLARVFRGEIMLPKARPGA

SEQ ID NO: 16 - protein, 772 aa, unidentified
  REGION 1..772: note = source = /note="Description of Unknown: anaerobic digester metagenome sequence"
MTRTKYREERTLVRGLQRLPNQDKTEFNKNVLRLRRHFEQFNLNVAELCQWLISFKPENPNSVCETKLFWEFMLEPENFCPDTYDRGSDWLRHEIFLLVAGWQTFEDMKAYNIRESLLTSAKMASSRPRSKTAEVLFIRLKSLEASHVMVLLKSASEWLSTRYIRQSENWKRHVQEWQKEKAAWEDKHPKLTPAIRDKYNAIFVELGISEKRSRVCSWKKLSENKDNCDWAGERKNIGDKWVSHSALCSKFNEFHRSLKGSPRKYFVTNANQYLELRRKNPQWTRDMAMQGLFRNVPGAQNWFPNAWTNYLNALNILETTILKDYNGHLPHCNKLSDECLFNQHTFNCRQYKRLLVGKLSSQERDLEETYREWRREYLAPPDKPFLRYPSAQKLPTPKLFGRGYYDLDFTRHVVKLRLDDMPAENFVSFGFKPWPRDYDKKPGEINITSVHVHFIGTRARVGFRFAVPHSYSRFSVSQDKIDELRSRVFPRKSQDLEFLNEARLRLLDGMNENQKSALRIMAVDLGTHRAAAAFFTGRIFDKPKLIKLKKIDLLTESITDTTQPEKHSANEKKIQREKGLTQHHVGKHLDTLETRTKEIISKRQNIKITPSDDTLGTLGDHDLRHLTSHIQRMIRDWVRLNAQQITELAEKEKVDLIVFESLRGFRAHAYDKLDLEQKRRLAFFAYGRIRRKVAEKAVERGMRVLTVPYFESSQICAQCGRSQNDKNKLRDNKRKQSFQCEFSDCNYKTHSDENAARVLGRVFWGEITLPTD

SEQ ID NO: 17 - protein, 696 aa, unidentified
  REGION 1..696: note = source = /note="Description of Unknown: aquatic-marine-marine sediment sequence"
MLEPERFCARNDPGDPRGDWIRHAVFEVVAGWKLSDNLDQYNLNEELTASIEAAMDKTRTATAEALFERLMRREASNVMVLLKVAAEWIAAKYVHQMENWKRQKEEWEKEKAEWENSHTELTEQVRDKYNRIFKELDIKNKRPRVCTWKRLSENKDNCDWAGKRKLIGKSWVNHAALCYKYHEYSEAPKVKHRDHFIANANKYIKIRREYPQWSRDQAMKTLFKNEPRASYWFPKEWKMYLGALGIEENTIIGNYTGCLPHCLKITHKCRFNKHTNECRRYKDLMHERLTNEERQLEELYREWRRNYLIAPGKPALRYPSARTLPTPKIFGSGYYRLDFERNQVHLRLDDMSQGDFISFGIKAWPRKYDYQPDTIDITSVQVHFVGTRARIGFRFKVPHRESIFTIRQDDIDELRSRKYPRESQDQKFLEEVRKRILNGFSEDQIAKLKIMAVDLGSDEGGVAFFKGHVFEKGESLKIIKIDELFESKKNEEAEKAKGLNVHHVGRHLDVLQKKSQEIALLRQGMTNAPSNDMVQSLYPNDMRRLTSHIRRMIRDWVRLNSSQIIKLAEREQVELIVFESMRGFLAPGYDKIDPDKKRRLAFFAFGSIRRKVAEKAVERGMRVVTVPYHCSSQVCAKCGKEQEDKKRFRKNKEKREFVCEDKKCNHKTNSDINAAHVCGRVFWGEINLLGKKIKIK

SEQ ID NO: 18 - protein, 768 aa, unidentified
  REGION 1..768: note = source = /note="Description of Unknown: aquatic-marine-marine sediment sequence"
MTRTKYREERTLVRSINRLPKQDKAEFKKNVLRLRRYFEQYNLDVSETCQWLISYRGLNLDEICKTQLFWEFMLEPERFCARNDPGDPRGDWIRHAVFEVVAGWKLSDNLDQYNLNEELTASIEAAMDKTRTATAEALFERLMRREASNVMVLLKVAAEWIAAKYVHQMENWKRQKEEWEKEKAEWENSHTELTEQVRDKYNRIFKELDIKNKRPRVCTWKRLSENKDNCDWAGKRKLIGKSWVNHAALCYKYHEYSEAPKVKHRDHFIANANKYIKIRREYPQWSRDQAMKTLFKNEPRASYWFPKEWKMYLGALGIEENTIIGNYTGCLPHCLKITHKCRFNKHTNECRRYKDLMHERLTNEERQLEELYREWRRNYLIAPGKPALRYPSARTLPTPKIFGSGYYRLDFERNQVHLRLDDMSQGDFISFGIKAWPRKYDYQPDTIDITSVQVHFVGTRARIGFRFKVPHRESIFTIRQDDIDELRSRKYPRESQDQKFLEEVRKRILNGFSEDQIAKLKIMAVDLGSDEGGVAFFKGHVFEKGESLKIIKIDELFESKKNEEAEKAKGLNVHHVGRHLDVLQKKSQEIALLRQGMTNAPSNDMVQSLYPNDMRRLTSHIRRMIRDWVRLNSSQIIKLAEREQVELIVFESMRGFLAPGYDKIDPDKKRRLAFFAFGSIRRKVAEKAVERGMRVVTVPYHCSSQVCAKCGKEQEDKKRFRKNKEKREFVCEDKKCNHKTNSDINAAHVCGRVFWGEINLLGKKIKIK

SEQ ID NO: 19 - protein, 855 aa, unidentified
  REGION 1..855: note = source = /note="Description of Unknown: aquatic-thermal springs-hot spring fe si sediment sequence"
MVASRYREARTLVRRLGRLPGEGEASFRAKLARLRKHFERFNVDVSELCQWLMGLRKQHCHKAGTASFGVLGDFLLHPESSNVAPGEAEADRWRLLVFDAVAGICPAKQLTNAPMPRGLPEAMEREAKRLADLEWRRRNTTQSKLIDRLAILEPAHRLVLLKAAAEWVVSRYQRGLENWAARRGEWEKERHAWEKRHPALSEEVRQRFTEVFKSLNDPERTDKPGVRRKNPRICPYERLRANIDNCIYAGEKGHGALCWKYAEFVKARKTRQPQFNDKRFAEDAEKVLPLLKQGMKRHQALQRLFPRDRPHGQLAQQRFNENWTAYLQALGLKEERVVNRGRLPHCLKIGETHEKSKCAWNPHTELCKQYKRALDQFDEETLKLEPLYREWRRDYLAGPGKPQFRYPSSRELPMPKIFGAGFHEIDFDRSILRLRLEDMPEGEWIEFGFAPWPRGYRPSKEEVKVKGAISSVHVNFVGVRARAGFRFDVRHRASRFQCTQDELDQLRSRAYPRRAQDREYLDAARKRLLESFAEGEEAAKRELRLLAVDLGETGACAAVYHGHAHQKDVQLAILKINRLYTQLPEALEPDPHGRPEEGKRKYERDDPRGVRKEHMGRHLKRMADGAASIAARRQGTMPATVTMAGHDFRGLKRHVTWMIRDWARHNAARIVAAAEEHGCDLIVFESLRGQKVPGYHELSSEKERDKRQLAMLSYGRIRHKVREKAVERGMRVVMVPDYRSSRLCSSCGHEQCAEKWQERRWRENKKKRLFKCVCGEPAPTEKPHHGGSAPDRQRAARRDGPGPGKRPGMAADQAKQRCRCGAEMNSDANAARVLARVFWGEITPPASERSFAGSA

SEQ ID NO: 20 - protein, 803 aa, unidentified
  REGION 1..803: note = source = /note="Description of Unknown: aquatic-thermal springs-hot spring fe si sediment sequence"
MGLRKQHCHKAGTASFGVLGDFLLHPESSNVAPGEAEADRWRLLVFDAVAGICPAKQLTNAPMPRGLPEAMEREAKRLADLEWRRRNTTQSKLIDRLAILEPAHRLVLLKAAAEWVVSRYQRGLENWAARRGEWEKERHAWEKRHPALSEEVRQRFTEVFKSLNDPERTDKPGVRRKNPRICPYERLRANIDNCIYAGEKGHGALCWKYAEFVKARKTRQPQFNDKRFAEDAEKVLPLLKQGMKRHQALQRLFPRDRPHGQLAQQRFNENWTAYLQALGLKEERVVNRGRLPHCLKIGETHEKSKCAWNPHTELCKQYKRALDQFDEETLKLEPLYREWRRDYLAGPGKPQFRYPSSRELPMPKIFGAGFHEIDFDRSILRLRLEDMPEGEWIEFGFAPWPRGYRPSKEEVKVKGAISSVHVNFVGVRARAGFRFDVRHRASRFQCTQDELDQLRSRAYPRRAQDREYLDAARKRLLESFAEGEEAAKRELRLLAVDLGETGACAAVYHGHAHQKDVQLAILKINRLYTQLPEALEPDPHGRPEEGKRKYERDDPRGVRKEHMGRHLKRMADGAASIAARRQGTMPATVTMAGHDFRGLKRHVTWMIRDWARHNAARIVAAAEEHGCDLIVFESLRGQKVPGYHELSSEKERDKRQLAMLSYGRIRHKVREKAVERGMRVVMVPDYRSSRLCSSCGHEQCAEKWQERRWRENKKKRLFKCVCGEPAPTEKPHHGGSAPDRQRAARRDGPGPGKRPGMAADQAKQRCRCGAEMNSDANAARVLARVFWGEITPPASERSFAGSA

SEQ ID NO: 21 - protein, 853 aa, unidentified
  REGION 1..853: note = source = /note="Description of Unknown: aquatic-thermal springs-sediment sequence"
MKNPKYREERTLTMGIRSFPLEDKSHFKEKVRKLRKFFEIFNKDVADLCQWLIVFRKGGKSENIPIWEFFINPLESIKDISEDQADELKRKVLDVIIGNESINNIRNEKLPTEVLKYLENLDDNWNQSVQELFKRMKDKKPSHRQILLKAASNLIYSRYYKTLENREKQKEEWKKERDTWQRKNPDLKEDIRTKYTEVYKQLGIKRKAPRICEWEKLKNWKHNCTYSSNKQHTERCFDFNKLFSSADNKKKRKWFIDNAHLYLQYLSKSNQKDALKQLYHKKKGSEKWFGRLWNDYLKLMKISEQDILTKYHCILPHCISENLGSAKYREYFDNSEYGFARSEFGKCANTYLGSRKKGSNKADSLQMVYGKHKSNIDERFEEIWNDYLKFIKKTEEEAIIEYNHSLPVYLKSDYCQFRPHGDKCKQYRDLLADFTEVEKSLEKKYREWRKSYLSGPGKPQFRYPSAKTIAIPKLFGSGYFRIDFEESILNLKLENDEWLSLGFKPWPKRKDYDIHYSDIEIPSVSIHFVGTRAKVGFRFKVKHKESRFKVAQEEIDKLRSQKYPRQYQDNDFLKEARELLLKDFDGDKNEMKILAFDWGETGAYAALFTGEKYEKGFQLPVLKFEKLYCSDKFKEAWDQKKKEQKWSKDESKAKLKEYKLKGLTKGHVGKHLENISEKAVKIAEIRGEKKDEKLLRPSDLRRLFSHSAWMIRDWVRLNTKQLIKIAEKNEVDLIVFESMRGSAPPSYDKLEEITEKIKWAFFSLGRIRHKVTEKAVERGMRTITVPYVKSSQVCFDCGKEAEDKKKWQHHKTELTKFICEHCPADLNSDENAARVLCKVFWGDITLPSTEWEK

SEQ ID NO: 22 - protein, 774 aa, unidentified
  REGION 1..774: note = source = /note="Description of Unknown: terrestrial-deep subsurface sequence"
MSNTRYSESRTLVRRLRRLPGESREEFRGKVRRLRKQFAQFNVNASELCQWLMSLRPGGKKASDRTKEFWEFFLEPERFLENQDDDRCDACRLAVFDVAAGLAPADRLGDYGVSQALAESVHVIGQISLTPTAAKLFTRLCGFEASHRQVLLKAAAEWIVAHYLRGYENWVRRHEEWEKEKARWEASHPELTQAARDDFNRIFKDLGIERKRPRVCTGERLKANKDDCDWAGERIPVGGTWRNHSSLCVKYWRFLKEYPRKARVPRQFREFFVTNAKTYMDLRRTSRGDRSVTMAAFLRKQRNAQWFPQAWEAYLKALEVNEQTVLAAGYGLPHCTEIGPDADCQFNKHTADCEKYRRALDARPDLLPLEKLYRHWRREYLSGPGKPCFQYPSQRKLPMPKIFGRGYFRVDLASSIIELRMEGGRDFERFRIAAWPSDYTPSAQEAQITSVHVSFVGTRALAGFRFEVPHKASRFAAGQDQIDELRSRKYPRRAQDAEFLVAARKRLLESFAGGAEHDVRILAVDLGTSNGAVAVFRGRSLEKAMPLDVIKLEKLHSSSPKENRGAGPEPSEEERKKARARGLRPSHVGRHLENWALAAREIANQRGNEADGPATLGDHDLRRFSLHIRWMIRDWVRLNVSQIIEAAEGNHVDLIVFESMRGWRAPGYDTVDDEKKRRLAFFAHGRIRHKIREKAVERGMRVVTVPYFMSSQFCGSCGTQQQDTRKLKTNKRERTSFTCENCGHRANSDENAAQVLAKVFWGDVVLPEDPDDCS

SEQ ID NO: 23 - protein, 763 aa, unidentified
  REGION 1..763: note = source = /note="Description of Unknown: terrestrial-deep subsurface sequence"
MVRRLRRLPGESREEFRGKVRRLRKQFAQFNVNASELCQWLMSLRPGGKKASDRTKEFWEFFLEPERFLENQDDDRCDACRLAVFDVAAGLAPADRLGDYGVSQALAESVHVIGQISLTPTAAKLFTRLCGFEASHRQVLLKAAAEWIVAHYLRGYENWVRRHEEWEKEKARWEASHPELTQAARDDFNRIFKDLGIERKRPRVCTGERLKANKDDCDWAGERIPVGGTWRNHSSLCVKYWRFLKEYPRKARVPRQFREFFVTNAKTYMDLRRTSRGDRSVTMAAFLRKQRNAQWFPQAWEAYLKALEVNEQTVLAAGYGLPHCTEIGPDADCQFNKHTADCEKYRRALDARPDLLPLEKLYRHWRREYLSGPGKPCFQYPSQRKLPMPKIFGRGYFRVDLASSIIELRMEGGRDFERFRIAAWPSDYTPSAQEAQITSVHVSFVGTRALAGFRFEVPHKASRFAAGQDQIDELRSRKYPRRAQDAEFLVAARKRLLESFAGGAEHDVRILAVDLGTSNGAVAVFRGRSLEKAMPLDVIKLEKLHSSSPKENRGAGPEPSEEERKKARARGLRPSHVGRHLENWALAAREIANQRGNEADGPATLGDHDLRRFSLHIRWMIRDWVRLNVSQIIEAAEGNHVDLIVFESMRGWRAPGYDTVDDEKKRRLAFFAHGRIRHKIREKAVERGMRVVTVPYFMSSQFCGSCGTQQQDTRKLKTNKRERTSFTCENCGHRANSDENAAQVLAKVFWGDVVLPEDPDDCS

SEQ ID NO: 24 - protein, 752 aa, unidentified
  REGION 1..752: note = source = /note="Description of Unknown: terrestrial-soil sequence"
MAVTRYREERTLVRGLRRLPGQSREQFRKNVLLLRRHFERFNVDVSDICQWMMGLRPKDGEVTPATQPLWDFMLEPSDGQGNAQGDPDRMRLLAFRVATGVEHSQSGVRLPLHVQESLRHVAALTSTESARRLILRFQQLEQSHQMILLKSASEWVRTRYSNANENWQRNRPLWEKEKAEWEKEHPALTPDACRKFSDIFKELGIKDKRPRICGWNRLKLPKDNCDYAGERVGGGRHAPLCKFYREFQAGLRREYKKQFPDNALKYLALRKQKGHTQAVVLQQFCAKDRRKSGWFPKAWMTYLQKLNVTEETLIQRYQGQLPHCVKIDNKTGCSFNPHTNDCLEYKKRILKLPESDRELETQYREWRRDYLSGPRKPSFRYPSSRNLPTPKIFGAGYYEADFTRSMLRLRLDDMPRGRFIEFGFKPWPSDYDIQPVSTQITSAHIHFIGTRARVGFRFAVAARPSRLRISQDEIDALRRQYPRAAQDQQFLDHVRPLILDSFAGNPKQELRILTIDLGTSGGAAAAFCGVTLVKSEVLKVIKLDKLYDLLDREDKRSPTSGLGEGHVGRHLEALSKEAAKIAQHRTTWKNPGLRPFDERQLTSHIRWMIRDWVRLNAQQIIEIAERENADLILFESMRGYYPKARDKYDSAQKVRLGFFSYGAIRRKVAEKAVERGMRILTLPYKFSSQICSKCGRKQENRGLKTKKAKRLFKCEHTGCGTELNSDENAARVLAGVFWGTIKLPEKAVVSHT

SEQ ID NO: 25 - DNA, 36 bp, synthetic construct
  misc_feature 1..36: note = source = /note="Description of Artificial Sequence: Synthetic oligonucleotide"
  source 1..36: mol_type = other DNA
ggtgcgaccggccgtcgattgaccggtttcgacacc

SEQ ID NO: 26 - DNA, 36 bp, synthetic construct
  misc_feature 1..36: note = source = /note="Description of Artificial Sequence: Synthetic oligonucleotide"
  source 1..36: mol_type = other DNA
gttgtagcgccccctgaattagcggtttccgacacc

SEQ ID NO: 27 - DNA, 36 bp, synthetic construct
  misc_feature 1..36: note = source = /note="Description of Artificial Sequence: Synthetic oligonucleotide"
  source 1..36: mol_type = other DNA
ggtgtaagtccgactgaatgcgaggtttccgacacc

SEQ ID NO: 28 - DNA, 36 bp, synthetic construct
  misc_feature 1..36: note = source = /note="Description of Artificial Sequence: Synthetic oligonucleotide"
  source 1..36: mol_type = other DNA
gctgtgactcaccggcatttgcggggttcttacacc

SEQ ID NO: 29 - DNA, 36 bp, synthetic construct
  misc_feature 1..36: note = source = /note="Description of Artificial Sequence: Synthetic oligonucleotide"
  source 1..36: mol_type = other DNA
gttgtgaccgcccccggaatcacggtttgcgacacc

SEQ ID NO: 30 - DNA, 36 bp, synthetic construct
  misc_feature 1..36: note = source = /note="Description of Artificial Sequence: Synthetic oligonucleotide"
  source 1..36: mol_type = other DNA
ggtgtagcgggcctcaaaaacacggcatccgacacc

SEQ ID NO: 31 - DNA, 46 bp, synthetic construct
  misc_feature 1..46: note = source = /note="Description of Artificial Sequence: Synthetic oligonucleotide"
  source 1..46: mol_type = other DNA
ggtttgcaaacagcgagaacatctgtgttttggtggtagttacaac

SEQ ID NO: 32 - DNA, 36 bp, synthetic construct
  misc_feature 1..36: note = source = /note="Description of Artificial Sequence: Synthetic oligonucleotide"
  source 1..36: mol_type = other DNA
gtttgcaaacagcgagaacatctgtgttttggtggt

SEQ ID NO: 33 - DNA, 36 bp, synthetic construct
  misc_feature 1..36: note = source = /note="Description of Artificial Sequence: Synthetic oligonucleotide"
  source 1..36: mol_type = other DNA
ggtggagccggccgtgaattagggggtttcgacacc

SEQ ID NO: 34 - DNA, 36 bp, synthetic construct
  misc_feature 1..36: note = source = /note="Description of Artificial Sequence: Synthetic oligonucleotide"
  source 1..36: mol_type = other DNA
ggtgttgtgaaccctgaaagaacggattccgacacc

SEQ ID NO: 35-102 - skipped (68 entries)

SEQ ID NO: 103 - DNA, 10 bp, synthetic construct
  misc_feature 1..10: note = source = /note="Description of Artificial Sequence: Synthetic oligonucleotide"
  source 1..10: mol_type = other DNA
ggtgtcggaa

SEQ ID NO: 104-112 - skipped (9 entries)

SEQ ID NO: 113 - DNA, 12 bp, synthetic construct
  misc_feature 1..12: note = source = /note="Description of Artificial Sequence: Synthetic oligonucleotide"
  source 1..12: mol_type = other DNA
gagccggtaaat

SEQ ID NO: 114-116 - skipped (3 entries)

SEQ ID NO: 117 - DNA, 159 bp, synthetic construct
  misc_feature 1..159: note = source = /note="Description of Artificial Sequence: Synthetic polynucleotide"
  source 1..159: mol_type = other DNA
tccgttcttctttgtagggtgttgtgaaccctgaaagaacggcgggtggcccggaccttggggcgtgttgaaaaacccgtttgtcgtcagttgatcggtgaaggttatcaagcgatggcgatcctgtagttgagatcgacggggttggtgtcagaccga

SEQ ID NO: 118 - DNA, 303 bp, synthetic construct
  misc_feature 1..303: note = source = /note="Description of Artificial Sequence: Synthetic polynucleotide"
  source 1..303: mol_type = other DNA
aacagcgacgaaaacgccgcacaggtgctggcgaaggtgttctggggcgacgtcgttctacccgaggatccggacgattgctcttgacgaagatatcgaaggtggtatagtgcccttgtgtcctcgtcgtgagtcgataatggctcggacaaaccccggcggagccttcggtgccaacgggaggaacctgagcccggaggatacaaactctctaattcgtggttgatatggcgatcaagaatgcggtttctttcaggcaattgtgtcgcaactctttgtcgatccagggattacgacgggaca

SEQ ID NO: 119 - DNA, 197 bp, synthetic construct
  misc_feature 1..197: note = source = /note="Description of Artificial Sequence: Synthetic polynucleotide"
  source 1..197: mol_type = other DNA
ccagacagcgaaaatgctgaataatcccggggacggcatacctaattgggttccagattgcccagcaggcagaagagagcgtttatcgcatttggggtgccggcggagagggggcgggccaagggtgtcactggatgtctccgctggtacccggcaaagcgtcaaacgcaatcaatcccggccgaaggccttccgct

SEQ ID NO: 120 - DNA, 310 bp, synthetic construct
  misc_feature 1..310: note = source = /note="Description of Artificial Sequence: Synthetic polynucleotide"
  source 1..310: mol_type = other DNA
agtacgcgggcacgcgggggcgtgtttagtacgcaggcacgcgggggcgtgtttagtacgcgggggcgtgattagtacaaaggggcaagtcaggtatacatcattaaagatgtcgaaaccgcaggggtttcgacctactcgaagaaagaaggtgtcggaacggcctgcatcatggggtttgggagggggattgggggctatttgaatcgaaacaaagttgatattgtccctatgcgggggattgtttgtagtgttgttcgagtaagaccaggttttcatcggggatgcggcctttttcaaaagagtcgac

SEQ ID NO: 121 - DNA, 191 bp, synthetic construct
  misc_feature 1..191: note = source = /note="Description of Artificial Sequence: Synthetic polynucleotide"
  source 1..191: mol_type = other DNA
cgagcgcgcgcttcagcacgaagcacgaggtgcggctgccggttgcattgcggcagaatgattggcccgcctgttcacgctttcccgaccggcagtggaaaacaaacgtcccgcacgtcgcagttcgtggcttagttgatgcgtgcgcgtgggccgattgacgggcgcgctcggctccgcctcgcggctaa

SEQ ID NO: 122 - DNA, 307 bp, synthetic construct
  misc_feature 1..307: note = source = /note="Description of Artificial Sequence: Synthetic polynucleotide"
  source 1..307: mol_type = other DNA
tttcgacacctgcgcaccgacttcaaagcaccatcggttgggtgcgaccggccgtcgattgaccggtttcgacaccccgctttgcacagcggcagcagacaaggatggtgcgaccggccgtcgattgaccggtttcgacaccactccgcctcgacggtcttaaccagttctgggtgcgaccggccgtcgattgaccggtttcgacaccctggacgtgtcgggcaatacttctgtcggaggtgcgaccggccgtcgattgaccggtttcgacacctacgccacggcaaagcacctgatcagctcgggt

SEQ ID NO: 123 - DNA, 307 bp, synthetic construct
  misc_feature 1..307: note = source = /note="Description of Artificial Sequence: Synthetic polynucleotide"
  source 1..307: mol_type = other DNA
tgctccactgggcgatgtatgcctgcaccactgggggtgctgcacgcggcggcgcagcgcctacaatggcgccgcggaaggggagcgcggcgcggtcatggaacccacgacgattgagatcaggaacgcgcgggagcataacctgcggtcggtgtcgctttcgttgccgcgggggaagctgattgtcttcaccggggtttcgggcagcgggaagagttcgctggcgtttgacacgctctatgccgaggggcagcggcggtatatcgagtcgttgtcgtcgtatgcccgacagttcatggggcagatg

SEQ ID NO: 124 - DNA, 307 bp, synthetic construct
  misc_feature 1..307: note = source = /note="Description of Artificial Sequence: Synthetic polynucleotide"
  source 1..307: mol_type = other DNA
tatgccgaggggcagcggcggtatatcgagtcgttgtcgtcgtatgcccgacagttcatggggcagatggccaagccggactgcgatcagatcacggggctttcgccatcgatcgcgattcagcagaagacgacgggatggaatccgcggtcgacggtggggacgacgacggcgatctatgactttctgcgcgtgctgtacgcgcggatcgggacgcagcattgcacgcagtgtgggcgggcgatcacggcgcagtctcgcgagcagatcgcggcggggatcttgagcgcgtttaatccgcgccgcg

SEQ ID NO: 125 - DNA, 307 bp, synthetic construct
  misc_feature 1..307: note = source = /note="Description of Artificial Sequence: Synthetic polynucleotide"
  source 1..307: mol_type = other DNA
ggcggtatatcgagtcgttgtcgtcgtatgcccgacagttcatggggcagatggccaagccggactgcgatcagatcacggggctttcgccatcgatcgcgattcagcagaagacgacgggatggaatccgcggtcgacggtggggacgacgacggcgatctatgactttctgcgcgtgctgtacgcgcggatcgggacgcagcattgcacgcagtgtgggcgggcgatcacggcgcagtctcgcgagcagatcgcggcggggatcttgagcgcgtttaatccgcgccgcgatcccacctatcagag

SEQ ID NO: 126 - DNA, 244 bp, synthetic construct
  misc_feature 1..244: note = source = /note="Description of Artificial Sequence: Synthetic polynucleotide"
  source 1..244: mol_type = other DNA
agccgacgagagcgcatttgccctccaaggcttgactctttttccagccgtggctacgctgttaatgcccttcgagtcgcattgtcctgcatacgcccggcggaacttcggtaccaacgggacggaccccggacacgaaaggcaaatgctgtgtttttgtggcctgccggtttggaacgtcacggttttgtgggcggttttttttgacgcaagtccttgtcagaagcgaatttgcagacgagac

SEQ ID NO: 127 - DNA, 173 bp, synthetic construct
  misc_feature 1..173: note = source = /note="Description of Artificial Sequence: Synthetic polynucleotide"
  source 1..173: mol_type = other DNA
ttcgagtcatttgcctggaatacgccctgcggacgttttcgaccaacgggatggacccctggcgctgaaggcagaatcggtttttcccgggcggtttcgggaggcgaacgagcggttttttcgaggtggaactggcgcaagtcgtgtccgttccggggcttgtttgccaagag

SEQ ID NO: 128 - DNA, 252 bp, synthetic construct
  misc_feature 1..252: note = source = /note="Description of Artificial Sequence: Synthetic polynucleotide"
  source 1..252: mol_type = other DNA
aattactctccccaccgattgatagttgaaaaaacttgacagacagcttaatttaagttatgtataatcagttgcttcgtggtccctctggccggaaaaacctctggcggagcgcaagcaccaatagagaggaactcggcccagaagcgaggaaaccgacaattaggggtttaattattgaaggaactttaaagattttgtgacggacggaataaattaagttcaaatcgcgtatgattatatgaatgatga

SEQ ID NO: 129 - DNA, 308 bp, synthetic construct
  misc_feature 1..308: note = source = /note="Description of Artificial Sequence: Synthetic polynucleotide"
  source 1..308: mol_type = other DNA
aaggtcgacaaagatttcggttggttataaatgaacgaggaggggcagatgtggacatctgccgcccacttgagtctggggcgataagctgattgtcgggggaggtttcaccaccgctggggggatcgatgtgaatcgtattgccgcctgggggccgcaataataaattaaacggcgtcaggaagaggttccagatgccgctcaatacccatagcacttagcccttgccttaacaatgaattgtgtctattttgagggctgtcttataaatagaaaagatatcaagataagttgtcgaaaccgcaggg

SEQ ID NO: 130 - DNA, 308 bp, synthetic construct
  misc_feature 1..308: note = source = /note="Description of Artificial Sequence: Synthetic polynucleotide"
  source 1..308: mol_type = other DNA
cctgggggccgcaataataaattaaacggcgtcaggaagaggttccagatgccgctcaatacccatagcacttagcccttgccttaacaatgaattgtgtctattttgagggctgtcttataaatagaaaagatatcaagataagttgtcgaaaccgcaggggtttcgacctaaaagaattatgtctgacgaagaaaaaaaagagaagaccaaatccgagatgccgtttctggatcatatcgaggaactgcgctggcggttgatcaagtccattttatcggttgccgtgatggccatcctggccttta

SEQ ID NO: 131 - DNA, 224 bp, synthetic construct
  misc_feature 1..224: note = source = /note="Description of Artificial Sequence: Synthetic polynucleotide"
  source 1..224: mol_type = other DNA
cgaaatcgagctgccgaccgcaatcccctgacgacccttgacggaactggccgatttgctaaaatatttttgatgcttacttagtcatctggttggcaaacctccgcggaccttcgggaccaatggagaggaacccagccgagaagcatcgagccggtaaatgccggaaatttttgagtcaggagaagctaacttcttcaaactcaggcccttggagccggtca

SEQ ID NO: 132 - DNA, 307 bp, synthetic construct
  misc_feature 1..307: note = source = /note="Description of Artificial Sequence: Synthetic polynucleotide"
  source 1..307: mol_type = other DNA
ctgtcctactgttttgacttaccgatgtgttactccaatacgggcggactgaagtccgccctccaggtgataatgatggagtttacgtctgcgtcacataaggacttgtgacgccaaatagctgtgattctacatcacgacggcagccggaatgccgccgctcccatgttgtaattcactggtgtttgtgattggagctcacgaataagaggtgggagaataaaaaaaactgccacttgcggacaggtggcagaacaaaattctccgaaacgcatgggttaaggctacctgcctgagggaacagaga

SEQ ID NO: 133 - DNA, 178 bp, synthetic construct
  misc_feature 1..178: note = source = /note="Description of Artificial Sequence: Synthetic polynucleotide"
  source 1..178: mol_type = other DNA
agttttgactggaaaatctccctttggacgtttgacctaggggagggaaccccgtctgaagatggataattaccgtcaaaatttggataaacttggagaaaattagacaaaagagtcggtttttttgatgttactgatcggcgtaactgatgtaactgtcgttagatacagcgagtcg

SEQ ID NO: 134 - DNA, 307 bp, synthetic construct
  misc_feature 1..307: note = source = /note="Description of Artificial Sequence: Synthetic polynucleotide"
  source 1..307: mol_type = other DNA
aataagaggaaacaatcctttcaatgtgagtttagtgactgtaattataaaacccatagcgatgagaatgcggcccgtgtcctcggacgggtattttggggtgaaattaccctccccaccgattgagtgttgaaaattcttgacatataggctaatttaagatatgtataattagtcgcttcgtggtccatctggccggaaaaacctctggcgggcgcaagcaccaatagagaggaactcggcccagaagcgaagaaaccaataattaggggtttaattattgaaggaactttaaagattttgcgac

SEQ ID NO: 135-149 - skipped (15 entries)

SEQ ID NO: 150 - RNA, 99 nt, synthetic construct
  variation 37..63: note = a, c, u, g, unknown or other
  misc_feature 1..99: note = source = /note="Description of Artificial Sequence: Synthetic oligonucleotide"
  source 1..99: mol_type = other RNA
gttgtagcgccccctgaattagcggtttccgacaccnnnnnnnnnnnnnnnnnnnnnnnnnnngttgtagcgccccctgaattagcggtttccgacacc

SEQ ID NO: 151 - RNA, 101 nt, synthetic construct
  variation 37..65: note = a, c, u, g, unknown or other
  misc_feature 1..101: note = source = /note="Description of Artificial Sequence: Synthetic polynucleotide"
  source 1..101: mol_type = other RNA
ggtgcggcagccggtagaactgcggcttccgacaccnnnnnnnnnnnnnnnnnnnnnnnnnnnnnggtgcggcagccggtagaactgcggcttccgacacc

SEQ ID NO: 152 - RNA, 101 nt, synthetic construct
  variation 37..65: note = a, c, u, g, unknown or other
  misc_feature 1..101: note = source = /note="Description of Artificial Sequence: Synthetic polynucleotide"
  source 1..101: mol_type = other RNA
ggtgtaagtccgactgaatgcgaggtttccgacaccnnnnnnnnnnnnnnnnnnnnnnnnnnnnnggtgtaagtccgactgaatgcgaggtttccgacacc

SEQ ID NO: 153 - RNA, 121 nt, synthetic construct
  variation 47..75: note = a, c, u, g, unknown or other
  misc_feature 1..121: note = source = /note="Description of Artificial Sequence: Synthetic polynucleotide"
  source 1..121: mol_type = other RNA
ggtttgcaaacagcgagaacatctgtgttttggtggtagttacaacnnnnnnnnnnnnnnnnnnnnnnnnnnnnnggtttgcaaacagcgagaacatctgtgttttggtggtagttacaac

SEQ ID NO: 154 - RNA, 101 nt, synthetic construct
  variation 37..65: note = a, c, u, g, unknown or other
  misc_feature 1..101: note = source = /note="Description of Artificial Sequence: Synthetic polynucleotide"
  source 1..101: mol_type = other RNA
gtttgcaaacagcgagaacatctgtgttttggtggtnnnnnnnnnnnnnnnnnnnnnnnnnnnnngtttgcaaacagcgagaacatctgtgttttggtggt

SEQ ID NO: 155 - RNA, 102 nt, synthetic construct
  variation 37..66: note = a, c, u, g, unknown or other
  misc_feature 1..102: note = source = /note="Description of Artificial Sequence: Synthetic polynucleotide"
  source 1..102: mol_type = other RNA
ggtggaaagggccggagatttaccggctctgacaccnnnnnnnnnnnnnnnnnnnnnnnnnnnnnnggtggaaagggccggagatttaccggctctgacacc

SEQ ID NO: 156 - RNA, 102 nt, synthetic construct; identical to SEQ ID NO: 155
  variation 37..66: note = a, c, u, g, unknown or other
  misc_feature 1..102: note = source = /note="Description of Artificial Sequence: Synthetic polynucleotide"
  source 1..102: mol_type = other RNA

SEQ ID NO: 157 - RNA, 102 nt, synthetic construct
  variation 37..66: note = a, c, u, g, unknown or other
  misc_feature 1..102: note = source = /note="Description of Artificial Sequence: Synthetic polynucleotide"
  source 1..102: mol_type = other RNA
ggtggagccggccgtgaattagggggtttcgacaccnnnnnnnnnnnnnnnnnnnnnnnnnnnnnnggtggagccggccgtgaattagggggtttcgacacc

SEQ ID NO: 158 - RNA, 102 nt, synthetic construct; identical to SEQ ID NO: 157
  variation 37..66: note = a, c, u, g, unknown or other
  misc_feature 1..102: note = source = /note="Description of Artificial Sequence: Synthetic polynucleotide"
  source 1..102: mol_type = other RNA

SEQ ID NO: 159 - RNA, 102 nt, synthetic construct
  variation 37..66: note = a, c, u, g, unknown or other
  misc_feature 1..102: note = source = /note="Description of Artificial Sequence: Synthetic polynucleotide"
  source 1..102: mol_type = other RNA
ggtgttgtgaaccctgaaagaacggattccgacaccnnnnnnnnnnnnnnnnnnnnnnnnnnnnnnggtgttgtgaaccctgaaagaacggattccgacacc

SEQ ID NO: 160 - RNA, 102 nt, synthetic construct
  variation 37..66: note = a, c, u, g, unknown or other
  misc_feature 1..102: note = source = /note="Description of Artificial Sequence: Synthetic polynucleotide"
  source 1..102: mol_type = other RNA
gttgtagcgccccctgaattagcggtttccgacaccnnnnnnnnnnnnnnnnnnnnnnnnnnnnnngttgtagcgccccctgaattagcggtttccgacacc

SEQ ID NO: 161 - RNA, 102 nt, synthetic construct
  variation 37..66: note = a, c, u, g, unknown or other
  misc_feature 1..102: note = source = /note="Description of Artificial Sequence: Synthetic polynucleotide"
  source 1..102: mol_type = other RNA
gttgtagcggcccctgaattagcggtttccgacaccnnnnnnnnnnnnnnnnnnnnnnnnnnnnnngttgtagcggcccctgaattagcggtttccgacacc

SEQ ID NO: 162 - RNA, 102 nt, synthetic construct
  variation 37..66: note = a, c, u, g, unknown or other
  misc_feature 1..102: note = source = /note="Description of Artificial Sequence: Synthetic polynucleotide"
  source 1..102: mol_type = other RNA
gttgtgaccgcccccggaatcacggtttgcgacaccnnnnnnnnnnnnnnnnnnnnnnnnnnnnnngttgtgaccgcccccggaatcacggtttgcgacacc

SEQ ID NO: 163 - RNA, 102 nt, synthetic construct; identical to SEQ ID NO: 162
  variation 37..66: note = a, c, u, g, unknown or other
  misc_feature 1..102: note = source = /note="Description of Artificial Sequence: Synthetic polynucleotide"
  source 1..102: mol_type = other RNA

SEQ ID NO: 164 - RNA, 104 nt, synthetic construct
  variation 37..68: note = a, c, u, g, unknown or other
  misc_feature 1..104: note = source = /note="Description of Artificial Sequence: Synthetic polynucleotide"
  source 1..104: mol_type = other RNA
ggtgtagcgggcctcaaaaacacggcatccgacaccnnnnnnnnnnnnnnnnnnnnnnnnnnnnnnnnggtgtagcgggcctcaaaaacacggcatccgacacc

SEQ ID NO: 165 - RNA, 104 nt, synthetic construct; identical to SEQ ID NO: 164
  variation 37..68: note = a, c, u, g, unknown or other
  misc_feature 1..104: note = source = /note="Description of Artificial Sequence: Synthetic polynucleotide"
  source 1..104: mol_type = other RNA

SEQ ID NO: 166 - RNA, 110 nt, synthetic construct
  variation 37..74: note = a, c, u, g, unknown or other
  misc_feature 1..110: note = source = /note="Description of Artificial Sequence: Synthetic polynucleotide"
  source 1..110: mol_type = other RNA
gctgtgactcaccggcatttgcggggttcttacaccnnnnnnnnnnnnnnnnnnnnnnnnnnnnnnnnnnnnnngctgtgactcaccggcatttgcggggttcttacacc

SEQ ID NO: 167 - RNA, 110 nt, synthetic construct; identical to SEQ ID NO: 166
  variation 37..74: note = a, c, u, g, unknown or other
  misc_feature 1..110: note = source = /note="Description of Artificial Sequence: Synthetic polynucleotide"
  source 1..110: mol_type = other RNA

SEQ ID NO: 168-199 - skipped (32 entries)

SEQ ID NO: 200 - DNA, 15 bp, synthetic construct
  variation 5: note = a, c, u, g, unknown or other
  misc_feature 1..15: note = source = /note="Description of Artificial Sequence: Synthetic oligonucleotide"
  misc_feature 1..15: note = source = /note="Description of Combined DNA/RNA Molecule: Synthetic oligonucleotide"
  source 1..15: mol_type = other DNA
rvsgnhtbbgacacc

SEQ ID NO: 201 - DNA, 15 bp, synthetic construct
  misc_feature 1..15: note = source = /note="Description of Artificial Sequence: Synthetic oligonucleotide"
  misc_feature 1..15: note = source = /note="Description of Combined DNA/RNA Molecule: Synthetic oligonucleotide"
  source 1..15: mol_type = other DNA
sgkggtwsttacamc

SEQ ID NO: 202 - RNA, 18 nt, synthetic construct
  misc_feature 1..18: note = source = /note="Description of Artificial Sequence: Synthetic oligonucleotide"
  source 1..18: mol_type = other RNA
tttaccggctctgacacc

SEQ ID NO: 203-209 - skipped (7 entries)

SEQ ID NO: 210 - protein, 5 aa, synthetic construct
  VARIANT 1: note = /replace="Gly" or "Ser" or Thr"
  VARIANT 2: note = /replace="Phe" or "Ile" or "Leu" or "Met" or "Pro" or "Val" "Trp" or "Tyr"
  VARIANT 4: note = /replace="Phe" or "Ile" or "Leu" or "Met" or "Pro" or "Val" "Trp" or "Tyr"
  VARIANT 5: note = /replace="Gly" or "Ser" or Thr"
  SITE 1..5: note = /note="Variant residues given in the sequence have no preference with respect to those in the annotations for variant positions"
  REGION 1..5: note = source = /note="Description of Artificial Sequence: Synthetic peptide"
ACDCA

SEQ ID NO: 211 - protein, 5 aa, synthetic construct
  VARIANT 1..4: note = /replace="Phe" or "Ile" or "Leu" or "Met" or "Pro" or "Val" "Trp" or "Tyr"
  SITE 1..5: note = /note="Variant residues given in the sequence have no preference with respect to those in the annotations for variant positions"
  REGION 1..5: note = source = /note="Description of Artificial Sequence: Synthetic peptide"
CCCCE

SEQ ID NO: 212 - protein, 5 aa, synthetic construct
  MOD_RES 2: note = Any amino acid
  REGION 1..5: note = source = /note="Description of Artificial Sequence: Synthetic peptide"
DXNAA

SEQ ID NO: 213-249 - skipped (37 entries)

SEQ ID NO: 250 - RNA, 99 nt, synthetic construct
  misc_feature 1..99: note = source = /note="Description of Artificial Sequence: Synthetic oligonucleotide"
  source 1..99: mol_type = other RNA
gatgcttacttagtcatctggttggcaaacctccgcggaccttcgggaccaatggagaggaacccagccgagaagcatcgagccggtaaatgccggaaa

SEQ ID NO: 251-299 - skipped (49 entries)

SEQ ID NO: 300 - protein, 7 aa, Simian virus 40
PKKKRKV

SEQ ID NO: 301 - protein, 16 aa, unidentified
  REGION 1..16: note = source = /note="Description of Unknown: Nucleoplasmin bipartite NLS sequence"
KRPAATKKAGQAKKKK

SEQ ID NO: 302 - protein, 9 aa, unidentified
  REGION 1..9: note = source = /note="Description of Unknown: c-Myc NLS sequence"
PAAKRVKLD

SEQ ID NO: 303 - protein, 11 aa, unidentified
  REGION 1..11: note = source = /note="Description of Unknown: c-Myc NLS sequence"
RQRRNELKRSP

SEQ ID NO: 304 - protein, 38 aa, Homo sapiens
NQSSNFGPMKGGNFGGRSSGPYGGGGQYFAKPRNQGGY

SEQ ID NO: 305 - protein, 42 aa, unidentified
  REGION 1..42: note = source = /note="Description of Unknown: IBB domain from importin-alpha sequence"
RMRIZFKNKGKDTAELRRRRVEVSVELRKAKKDEQILKRRNV

SEQ ID NO: 306 - protein, 8 aa, unidentified
  REGION 1..8: note = source = /note="Description of Unknown: Myoma T protein sequence"
VSRKRPRP

SEQ ID NO: 307 - protein, 8 aa, unidentified
  REGION 1..8: note = source = /note="Description of Unknown: Myoma T protein sequence"
PPKKARED

SEQ ID NO: 308 - protein, 8 aa, Homo sapiens
PQPKKKPL

SEQ ID NO: 309 - protein, 12 aa, Mus sp.
SALIKKKKKMAP

SEQ ID NO: 310 - protein, 5 aa, Influenza virus
DRLRR

SEQ ID NO: 311 - protein, 7 aa, Influenza virus
PKQKKRK

SEQ ID NO: 312 - protein, 10 aa, Mus sp.
RKLKKKIKKL

SEQ ID NO: 313 - protein, 10 aa, Mus sp.
REKKKFLKRR

SEQ ID NO: 314 - protein, 20 aa, Homo sapiens
KRKGDEVDGVDEVAKKKSKK

SEQ ID NO: 315 - protein, 17 aa, Homo sapiens
RKCLQAGMNLEARKTKK

SEQ ID NO: 316 - protein, 130 aa, synthetic construct
  REGION 1..130: note = source = /note="Description of Artificial Sequence: Synthetic polypeptide"
MASNFTQFVLVDNGGTGDVTVAPSNFANGVAEWISSNSRSQAYKVTCSVRQSSAQKRKYTIKVEVPKVATQTVGGVELPVAAWRSYLNMELTIPIFATNSDCELIVKAMQGLLKDGNPIPSAIAANSGIY

SEQ ID NO: 317 - protein, 133 aa, synthetic construct
  REGION 1..133: note = source = /note="Description of Artificial Sequence: Synthetic polypeptide"
MAKLETVTLGNIGKDGKQTLVLNPRGVNPTNGVASLSQAGAVPALEKRVTVSVSQPSRNRKNYKVQVKIQNPTACTANGSCDPSVTRQAYADVTFSFTQYSTDEERAFVRTELAALLASPLLIDAIDQLNPAY

SEQ ID NO: 318 - protein, 128 aa, synthetic construct
  REGION 1..128: note = source = /note="Description of Artificial Sequence: Synthetic polypeptide"
MSKTIVLSVGEATRTLTEIQSTADRQIFEEKVGPLVGRLRLTASLRQNGAKTAYRVNLKLDQADVVDCSTSVCGELPKVRYTQVWSHDVTIVANSTEASRKSLYDLTKSLVVQATSEDLVVNLVPLGR

SEQ ID NO: 319-399 - skipped (81 entries)

SEQ ID NO: 400 - RNA, 171 nt, synthetic construct
  misc_feature 1..171: note = source = /note="Description of Artificial Sequence: Synthetic polynucleotide"
  source 1..171: mol_type = other RNA
gggggtggaaagggccggagatttaccggctctgacaccccattcatccgcttattatcacttattcagggtggaaagggccggagatttaccggctctgacaccgcttggaggagcgcagtcaccaaaacttgtggtggaaagggccggagatttaccggctctgacacc

SEQ ID NO: 401 - RNA, 36 nt, synthetic construct
  misc_feature 1..36: note = source = /note="Description of Artificial Sequence: Synthetic oligonucleotide"
  source 1..36: mol_type = other RNA
ggtggaaagggccggagatttaccggctctgacacc

SEQ ID NO: 402 - RNA, 30 nt, synthetic construct
  misc_feature 1..30: note = source = /note="Description of Artificial Sequence: Synthetic oligonucleotide"
  source 1..30: mol_type = other RNA
ccattcatccgcttattatcacttattcag

SEQ ID NO: 403 - RNA, 30 nt, synthetic construct
  misc_feature 1..30: note = source = /note="Description of Artificial Sequence: Synthetic oligonucleotide"
  source 1..30: mol_type = other RNA
gcttggaggagcgcagtcaccaaaacttgt

SEQ ID NO: 404 - RNA, 107 nt, synthetic construct
  misc_feature 1..107: note = source = /note="Description of Artificial Sequence: Synthetic polynucleotide"
  source 1..107: mol_type = other RNA
ggggatgcttacttagtcatctggttggcaaacctccgcggaccttcgggaccaatggagaggaacccagccgagaagcatcgagccggtaaatgccggaaattttt

SEQ ID NO: 405 - RNA, 102 nt, synthetic construct
  misc_feature 1..102: note = source = /note="Description of Artificial Sequence: Synthetic polynucleotide"
  source 1..102: mol_type = other RNA
ggggatgcttacttagtcatctggttggcaaacctccgcggaccttcgggaccaatggagaggaacccagccgagaagcatcgagccggtaaatgccggaaa

SEQ ID NO: 406 - RNA, 94 nt, synthetic construct
  misc_feature 1..94: note = source = /note="Description of Artificial Sequence: Synthetic oligonucleotide"
  source 1..94: mol_type = other RNA
ggggatgcttacttagtcatctggttggcaaacctccgcggaccttcgggaccaatggagaggaacccagccgagaagcatcgagccggtaaat

SEQ ID NO: 407 - RNA, 45 nt, synthetic construct
  misc_feature 1..45: note = source = /note="Description of Artificial Sequence: Synthetic oligonucleotide"
  source 1..45: mol_type = other RNA
gggtttaccggctctgacaccgcttggaggagcgcagtcaccaaa

SEQ ID NO: 408 - RNA, 18 nt, synthetic construct
  misc_feature 1..18: note = source = /note="Description of Artificial Sequence: Synthetic oligonucleotide"
  source 1..18: mol_type = other RNA
tttaccggctctgacacc

SEQ ID NO: 409 - RNA, 24 nt, synthetic construct
  misc_feature 1..24: note = source = /note="Description of Artificial Sequence: Synthetic oligonucleotide"
  source 1..24: mol_type = other RNA
gcttggaggagcgcagtcaccaaa

SEQ ID NO: 410 - RNA, 45 nt, synthetic construct
  misc_feature 1..45: note = source = /note="Description of Artificial Sequence: Synthetic oligonucleotide"
  source 1..45: mol_type = other RNA
gggtttaccggctctgacaccaactgtgataaactaccgcattaa

SEQ ID NO: 411 - RNA, 18 nt, synthetic construct
  misc_feature 1..18: note = source = /note="Description of Artificial Sequence: Synthetic oligonucleotide"
  source 1..18: mol_type = other RNA
tttaccggctctgacacc

SEQ ID NO: 412 - RNA, 24 nt, synthetic construct
  misc_feature 1..24: note = source = /note="Description of Artificial Sequence: Synthetic oligonucleotide"
  source 1..24: mol_type = other RNA
aactgtgataaactaccgcattaa

SEQ ID NO: 413 - RNA, 45 nt, synthetic construct
  misc_feature 1..45: note = source = /note="Description of Artificial Sequence: Synthetic oligonucleotide"
  source 1..45: mol_type = other RNA
gggtttaccggctctgacacccttccttagctcctgaaaatctcg

SEQ ID NO: 414 - RNA, 18 nt, synthetic construct
  misc_feature 1..18: note = source = /note="Description of Artificial Sequence: Synthetic oligonucleotide"
  source 1..18: mol_type = other RNA
tttaccggctctgacacc

SEQ ID NO: 415 - RNA, 24 nt, synthetic construct
  misc_feature 1..24: note = source = /note="Description of Artificial Sequence: Synthetic oligonucleotide"
  source 1..24: mol_type = other RNA
cttccttagctcctgaaaatctcg

SEQ ID NO: 416 - RNA, 45 nt, synthetic construct
  misc_feature 1..45: note = source = /note="Description of Artificial Sequence: Synthetic oligonucleotide"
  source 1..45: mol_type = other RNA
gggtttaccggctctgacacccatcttgcgaatatatgtgtagaa

SEQ ID NO: 417 - RNA, 18 nt, synthetic construct
  misc_feature 1..18: note = source = /note="Description of Artificial Sequence: Synthetic oligonucleotide"
  source 1..18: mol_type = other RNA
tttaccggctctgacacc

SEQ ID NO: 418 - RNA, 24 nt, synthetic construct
  misc_feature 1..24: note = source = /note="Description of Artificial Sequence: Synthetic oligonucleotide"
  source 1..24: mol_type = other RNA
catcttgcgaatatatgtgtagaa

SEQ ID NO: 419 - RNA, 130 nt, synthetic construct
  misc_feature 1..130: note = source = /note="Description of Artificial Sequence: Synthetic polynucleotide"
  source 1..130: mol_type = other RNA
caacgaggtatttatccgattaattctcatgtttgacagcttatcatcgataagctttaatgcggtagtttatcacagttaaattgctaacgcagtcaggcaccgtgtatttgtagcccggggactgttt

SEQ ID NO: 420 - RNA, 130 nt, synthetic construct
  misc_feature 1..130: note = source = /note="Description of Artificial Sequence: Synthetic polynucleotide"
  source 1..130: mol_type = other RNA
caacgaggtatttatccgataaataagatcactaccgggcgtattttttgagttatcgagattttcaggagctaaggaagctaaaatggagaaaaaaatcactggatatattgtagcccggggactgttt

SEQ ID NO: 421 - RNA, 130 nt, synthetic construct; identical to SEQ ID NO: 419
  misc_feature 1..130: note = source = /note="Description of Artificial Sequence: Synthetic polynucleotide"
  source 1..130: mol_type = other RNA

SEQ ID NO: 422 - DNA, 130 bp, synthetic construct
  misc_feature 1..130: note = source = /note="Description of Artificial Sequence: Synthetic polynucleotide"
  source 1..130: mol_type = other DNA
caacgaggtatttatccgattaattctcatgtttgacagcttatcatcgataagctttaatgcggtagtttatcacagttaaattgctaacgcagtcaggcaccgtgtatttgtagcccggggactgttt

SEQ ID NO: 423 - RNA, 130 nt, synthetic construct
  misc_feature 1..130: note = source = /note="Description of Artificial Sequence: Synthetic polynucleotide"
  source 1..130: mol_type = other RNA
aaacagtccccgggctacaaatacacggtgcctgactgcgttagcaatttaactgtgataaactaccgcattaaagcttatcgatgataagctgtcaaacatgagaattaatcggataaatacctcgttg

SEQ ID NO: 424 - DNA, 130 bp, synthetic construct
  misc_feature 1..130: note = source = /note="Description of Artificial Sequence: Synthetic polynucleotide"
  source 1..130: mol_type = other DNA
aaacagtccccgggctacaaatacacggtgcctgactgcgttagcaatttaactgtgataaactaccgcattaaagcttatcgatgataagctgtcaaacatgagaattaatcggataaatacctcgttg

SEQ ID NO: 425 - DNA, 130 bp, synthetic construct
  misc_feature 1..130: note = source = /note="Description of Artificial Sequence: Synthetic polynucleotide"
  source 1..130: mol_type = other DNA
caacgaggtatttatccgatcgctctggagtgaataccacgacgatttccggcagtttctacacatatattcgcaagatgtggcgtgttacggtgaaaacctggcctattttgtagcccggggactgttt

SEQ ID NO: 426 - RNA, 130 nt, synthetic construct; identical to SEQ ID NO: 423
  misc_feature 1..130: note = source = /note="Description of Artificial Sequence: Synthetic polynucleotide"
  source 1..130: mol_type = other RNA

SEQ ID NO: 427 - RNA, 130 nt, synthetic construct
  misc_feature 1..130: note = source = /note="Description of Artificial Sequence: Synthetic polynucleotide"
  source 1..130: mol_type = other RNA
aaacagtccccgggctacaatatatccagtgatttttttctccattttagcttccttagctcctgaaaatctcgataactcaaaaaatacgcccggtagtgatcttatttatcggataaatacctcgttg

SEQ ID NO: 428 - RNA, 130 nt, synthetic construct
  misc_feature 1..130: note = source = /note="Description of Artificial Sequence: Synthetic polynucleotide"
  source 1..130: mol_type = other RNA
aaacagtccccgggctacaatctcgccgaaacgtttggtggcgggaccagtgacgaaggcttgagcgagggcgtgcaagattccgaataccgcaagcgacaggccgatcaatcggataaatacctcgttg

SEQ ID NO: 429 - DNA, 130 bp, synthetic construct
  misc_feature 1..130: note = source = /note="Description of Artificial Sequence: Synthetic polynucleotide"
  source 1..130: mol_type = other DNA
aaacagtccccgggctacaaaataggccaggttttcaccgtaacacgccacatcttgcgaatatatgtgtagaaactgccggaaatcgtcgtggtattcactccagagcgatcggataaatacctcgttg

SEQ ID NO: 430 - DNA, 188 bp, synthetic construct
  misc_feature 1..188: note = source = /note="Description of Artificial Sequence: Synthetic polynucleotide"
  source 1..188: mol_type = other DNA
ggtgtcagagccggtaaatctccggccctttccaccacaagttttggtgactgcgctcctccaagcggtgtcagagccggtaaatctccggccctttccaccctgaataagtgataataagcggatgaatggggtgtcagagccggtaaatctccggccctttccaccccctatagtgagtcgtatta

SEQ ID NO: 431 - DNA, 18 bp, synthetic construct
  misc_feature 1..18: note = source = /note="Description of Artificial Sequence: Synthetic oligonucleotide"
  source 1..18: mol_type = other DNA
taatacgactcactatag

SEQ ID NO: 432 - DNA, 66 bp, synthetic construct
  misc_feature 1..66: note = source = /note="Description of Artificial Sequence: Synthetic oligonucleotide"
  source 1..66: mol_type = other DNA
ggtgtcagagccggtaaatctccggccctttccaccacaagttttggtgactgcgctcctccaagc

SEQ ID NO: 433 - DNA, 124 bp, synthetic construct
  misc_feature 1..124: note = source = /note="Description of Artificial Sequence: Synthetic polynucleotide"
  source 1..124: mol_type = other DNA
ttaatgcggtagtttatcacagttggtgtcagagccggtaaaccctatagtgagtcgtattattaatgcggtagtttatcacagttggtgtcagagccggtaaaccctatagtgagtcgtatta

SEQ ID NO: 434 - DNA, 36 bp, synthetic construct
  misc_feature 1..36: note = source = /note="Description of Artificial Sequence: Synthetic oligonucleotide"
  source 1..36: mol_type = other DNA
taatacgactcactatagtaatacgactcactatag

SEQ ID NO: 435 - DNA, 124 bp, synthetic construct
  misc_feature 1..124: note = source = /note="Description of Artificial Sequence: Synthetic polynucleotide"
  source 1..124: mol_type = other DNA
cgagattttcaggagctaaggaagggtgtcagagccggtaaaccctatagtgagtcgtattacgagattttcaggagctaaggaagggtgtcagagccggtaaaccctatagtgagtcgtatta

SEQ ID NO: 436 - DNA, 36 bp, synthetic construct; identical to SEQ ID NO: 434
  misc_feature 1..36: note = source = /note="Description of Artificial Sequence: Synthetic oligonucleotide"
  source 1..36: mol_type = other DNA

SEQ ID NO: 437 - DNA, 124 bp, synthetic construct
  misc_feature 1..124: note = source = /note="Description of Artificial Sequence: Synthetic polynucleotide"
  source 1..124: mol_type = other DNA
ttctacacatatattcgcaagatgggtgtcagagccggtaaaccctatagtgagtcgtattattctacacatatattcgcaagatgggtgtcagagccggtaaaccctatagtgagtcgtatta

SEQ ID NO: 438 - DNA, 36 bp, synthetic construct; identical to SEQ ID NO: 434
  misc_feature 1..36: note = source = /note="Description of Artificial Sequence: Synthetic oligonucleotide"
  source 1..36: mol_type = other DNA

SEQ ID NO: 439 - DNA, 248 bp, synthetic construct
  misc_feature 1..248: note = source = /note="Description of Artificial Sequence: Synthetic polynucleotide"
  source 1..248: mol_type = other DNA
aaaaatttccggcatttaccggctcgatgcttctcggctgggttcctctccattggtcccgaaggtccgcggaggtttgccaaccagatgactaagtaagcatcccctatagtgagtcgtattaaaaaatttccggcatttaccggctcgatgcttctcggctgggttcctctccattggtcccgaaggtccgcggaggtttgccaaccagatgactaagtaagcatcccctatagtgagtcgtatta

SEQ ID NO: 440 - DNA, 36 bp, synthetic construct; identical to SEQ ID NO: 434
  misc_feature 1..36: note = source = /note="Description of Artificial Sequence: Synthetic oligonucleotide"
  source 1..36: mol_type = other DNA

SEQ ID NO: 441 - DNA, 238 bp, synthetic construct
  misc_feature 1..238: note = source = /note="Description of Artificial Sequence: Synthetic polynucleotide"
  source 1..238: mol_type = other DNA
tttccggcatttaccggctcgatgcttctcggctgggttcctctccattggtcccgaaggtccgcggaggtttgccaaccagatgactaagtaagcatcccctatagtgagtcgtattatttccggcatttaccggctcgatgcttctcggctgggttcctctccattggtcccgaaggtccgcggaggtttgccaaccagatgactaagtaagcatcccctatagtgagtcgtatta

SEQ ID NO: 442 - DNA, 36 bp, synthetic construct; identical to SEQ ID NO: 434
  misc_feature 1..36: note = source = /note="Description of Artificial Sequence: Synthetic oligonucleotide"
  source 1..36: mol_type = other DNA

SEQ ID NO: 443 - DNA, 222 bp, synthetic construct
  misc_feature 1..222: note = source = /note="Description of Artificial Sequence: Synthetic polynucleotide"
  source 1..222: mol_type = other DNA
atttaccggctcgatgcttctcggctgggttcctctccattggtcccgaaggtccgcggaggtttgccaaccagatgactaagtaagcatcccctatagtgagtcgtattaatttaccggctcgatgcttctcggctgggttcctctccattggtcccgaaggtccgcggaggtttgccaaccagatgactaagtaagcatcccctatagtgagtcgtatta

SEQ ID NO: 444 - DNA, 36 bp, synthetic construct; identical to SEQ ID NO: 434
  misc_feature 1..36: note = source = /note="Description of Artificial Sequence: Synthetic oligonucleotide"
  source 1..36: mol_type = other DNA

SEQ ID NO: 445 - DNA, 130 bp, synthetic construct
  misc_feature 1..130: note = source = /note="Description of Artificial Sequence: Synthetic polynucleotide"
  source 1..130: mol_type = other DNA
aaacagtccccgggctacaaagctaccaactctttgaaccgaggtaactggcttggaggagcgcagtcaccaaaacttgtcctttcagtttagccttaaccggcgcatgaatcggataaatacctcgttg

SEQ ID NO: 446 - DNA, 20 bp, synthetic construct
  misc_feature 1..20: note = source = /note="Description of Artificial Sequence: Synthetic oligonucleotide"
  source 1..20: mol_type = other DNA
aaacagtccccgggctacaa

SEQ ID NO: 447 - DNA, 63 bp, synthetic construct
  misc_feature 1..63: note = source = /note="Description of Artificial Sequence: Synthetic oligonucleotide"
  source 1..63: mol_type = other DNA
aaatgtaataaggatccctcgagtaatacgactcactatagggcaacgaggtatttatccgat

SEQ ID NO: 448 - DNA, 63 bp, synthetic construct
  misc_feature 1..63: note = source = /note="Description of Artificial Sequence: Synthetic oligonucleotide"
  source 1..63: mol_type = other DNA
aaatgtaataaggatccctcgagtaatacgactcactatagggaaacagtccccgggctacaa

SEQ ID NO: 449 - DNA, 20 bp, synthetic construct
  misc_feature 1..20: note = source = /note="Description of Artificial Sequence: Synthetic oligonucleotide"
  source 1..20: mol_type = other DNA
caacgaggtatttatccgat

SEQ ID NO: 450 - DNA, 130 bp, synthetic construct; identical to SEQ ID NO: 424
  misc_feature 1..130: note = source = /note="Description of Artificial Sequence: Synthetic polynucleotide"
  source 1..130: mol_type = other DNA

SEQ ID NO: 451 - DNA, 20 bp, synthetic construct
  misc_feature 1..20: note = source = /note="Description of Artificial Sequence: Synthetic oligonucleotide"
  source 1..20: mol_type = other DNA
aaacagtccccgggctacaa

SEQ ID NO: 452 - DNA, 63 bp, synthetic construct; identical to SEQ ID NO: 447
  misc_feature 1..63: note = source = /note="Description of Artificial Sequence: Synthetic oligonucleotide"
  source 1..63: mol_type = other DNA

SEQ ID NO: 453 - DNA, 63 bp, synthetic construct; identical to SEQ ID NO: 448
  misc_feature 1..63: note = source = /note="Description of Artificial Sequence: Synthetic oligonucleotide"
  source 1..63: mol_type = other DNA

SEQ ID NO: 454 - DNA, 20 bp, synthetic construct
  misc_feature 1..20: note = source = /note="Description of Artificial Sequence: Synthetic oligonucleotide"
  source 1..20: mol_type = other DNA
caacgaggtatttatccgat

SEQ ID NO: 455 - DNA, 130 bp, synthetic construct
  misc_feature 1..130: note = source = /note="Description of Artificial Sequence: Synthetic polynucleotide"
  source 1..130: mol_type = other DNA
aaacagtccccgggctacaatatatccagtgatttttttctccattttagcttccttagctcctgaaaatctcgataactcaaaaaatacgcccggtagtgatcttatttatcggataaatacctcgttg

SEQ ID NO: 456 - DNA, 20 bp, synthetic construct
  misc_feature 1..20: note = source = /note="Description of Artificial Sequence: Synthetic oligonucleotide"
  source 1..20: mol_type = other DNA
aaacagtccccgggctacaa

SEQ ID NO: 457 - DNA, 63 bp, synthetic construct; identical to SEQ ID NO: 447
  misc_feature 1..63: note = source = /note="Description of Artificial Sequence: Synthetic oligonucleotide"
  source 1..63: mol_type = other DNA

SEQ ID NO: 458 - DNA, 63 bp, synthetic construct; identical to SEQ ID NO: 448
  misc_feature 1..63: note = source = /note="Description of Artificial Sequence: Synthetic oligonucleotide"
  source 1..63: mol_type = other DNA

SEQ ID NO: 459 - DNA, 20 bp, synthetic construct
  misc_feature 1..20: note = source = /note="Description of Artificial Sequence: Synthetic oligonucleotide"
  source 1..20: mol_type = other DNA
caacgaggtatttatccgat

SEQ ID NO: 460 - DNA, 130 bp, synthetic construct; identical to SEQ ID NO: 429
  misc_feature 1..130: note = source = /note="Description of Artificial Sequence: Synthetic polynucleotide"
  source 1..130: mol_type = other DNA

SEQ ID NO: 461 - DNA, 20 bp, synthetic construct
  misc_feature 1..20: note = source = /note="Description of Artificial Sequence: Synthetic oligonucleotide"
  source 1..20: mol_type = other DNA
aaacagtccccgggctacaa

SEQ ID NO: 462 - DNA, 63 bp, synthetic construct; identical to SEQ ID NO: 447
  misc_feature 1..63: note = source = /note="Description of Artificial Sequence: Synthetic oligonucleotide"
  source 1..63: mol_type = other DNA

SEQ ID NO: 463 - DNA, 63 bp, synthetic construct; identical to SEQ ID NO: 448
  misc_feature 1..63: note = source = /note="Description of Artificial Sequence: Synthetic oligonucleotide"
  source 1..63: mol_type = other DNA

SEQ ID NO: 464 - DNA, 20 bp, synthetic construct
  misc_feature 1..20: note = source = /note="Description of Artificial Sequence: Synthetic oligonucleotide"
  source 1..20: mol_type = other DNA
caacgaggtatttatccgat

SEQ ID NO: 465 - DNA, 130 bp, synthetic construct
  misc_feature 1..130: note = source = /note="Description of Artificial Sequence: Synthetic polynucleotide"
  source 1..130: mol_type = other DNA
aaacagtccccgggctacaatctcgccgaaacgtttggtggcgggaccagtgacgaaggcttgagcgagggcgtgcaagattccgaataccgcaagcgacaggccgatcaatcggataaatacctcgttg

SEQ ID NO: 466 - DNA, 20 bp, synthetic construct
  misc_feature 1..20: note = source = /note="Description of Artificial Sequence: Synthetic oligonucleotide"
  source 1..20: mol_type = other DNA
aaacagtccccgggctacaa

SEQ ID NO: 467 - DNA, 63 bp, synthetic construct; identical to SEQ ID NO: 447
  misc_feature 1..63: note = source = /note="Description of Artificial Sequence: Synthetic oligonucleotide"
  source 1..63: mol_type = other DNA

SEQ ID NO: 468 - DNA, 63 bp, synthetic construct; identical to SEQ ID NO: 448
  misc_feature 1..63: note = source = /note="Description of Artificial Sequence: Synthetic oligonucleotide"
  source 1..63: mol_type = other DNA

SEQ ID NO: 469 - DNA, 20 bp, synthetic construct
  misc_feature 1..20: note = source = /note="Description of Artificial Sequence: Synthetic oligonucleotide"
  source 1..20: mol_type = other DNA
caacgaggtatttatccgat

SEQ ID NO: 470 - RNA, 36 nt, synthetic construct
  misc_feature 1..36: note = source = /note="Description of Artificial Sequence: Synthetic oligonucleotide"
  source 1..36: mol_type = other RNA
gttgtagcggcccctgaattagcggtttccgacacc

SEQ ID NO: 471 - RNA, 36 nt, synthetic construct
  misc_feature 1..36: note = source = /note="Description of Artificial Sequence: Synthetic oligonucleotide"
  source 1..36: mol_type = other RNA
ggtgcggcagccggtagaactgcggcttccgacacc

SEQ ID NO: 472 - RNA, 36 nt, synthetic construct
  misc_feature 1..36: note = source = /note="Description of Artificial Sequence: Synthetic oligonucleotide"
  source 1..36: mol_type = other RNA
gttggagtcagcaaggaatcaacggttttggacacc

SEQ ID NO: 473 - RNA, 34 nt, synthetic construct
  misc_feature 1..34: note = source = /note="Description of Artificial Sequence: Synthetic oligonucleotide"
  source 1..34: mol_type = other RNA
ggtgtagcgggcctcaaaaacacggcatccgaca

SEQ ID NO: 474 - RNA, 28 nt, synthetic construct
  misc_feature 1..28: note = source = /note="Description of Artificial Sequence: Synthetic oligonucleotide"
  source 1..28: mol_type = other RNA
gctgtgactcaccggcatttgcggggtt

SEQ ID NO: 475 - DNA, 102 bp, synthetic construct
  variation 37..66: note = a, c, u, g, unknown or other
  misc_feature 1..102: note = source = /note="Description of Artificial Sequence: Synthetic polynucleotide"
  source 1..102: mol_type = other DNA
ggtggaaagggccggagatttaccggctctgacaccnnnnnnnnnnnnnnnnnnnnnnnnnnnnnnggtggaaagggccggagatttaccggctctgacacc

SEQ ID NO: 476 - RNA, 39 nt, synthetic construct
  variation 19..39: note = a, c, u, g, unknown or other
  misc_feature 1..39: note = source = /note="Description of Artificial Sequence: Synthetic oligonucleotide"
  source 1..39: mol_type = other RNA
tttaccggctctgacaccnnnnnnnnnnnnnnnnnnnnn

SEQ ID NO: 477 - DNA, 36 bp, synthetic construct
  misc_feature 1..36: note = source = /note="Description of Artificial Sequence: Synthetic oligonucleotide"
  source 1..36: mol_type = other DNA
cgataagctttaatgcggtagtttatcacagttaaa

SEQ ID NO: 478 - RNA, 36 nt, synthetic construct
  misc_feature 1..36: note = source = /note="Description of Artificial Sequence: Synthetic oligonucleotide"
  source 1..36: mol_type = other RNA
cgataagctttaatgcggtagtttatcacagttaaa

SEQ ID NO: 479 - RNA, 36 nt, synthetic construct
  misc_feature 1..36: note = source = /note="Description of Artificial Sequence: Synthetic oligonucleotide"
  source 1..36: mol_type = other RNA
tttaactgtgataaactaccgcattaaagcttatcg

SEQ ID NO: 480 - DNA, 36 bp, synthetic construct
  misc_feature 1..36: note = source = /note="Description of Artificial Sequence: Synthetic oligonucleotide"
  source 1..36: mol_type = other DNA
tttaactgtgataaactaccgcattaaagcttatcg

SEQ ID NO: 481 - protein, 5 aa, synthetic construct
  REGION 1..5: note = source = /note="Description of Artificial Sequence: Synthetic peptide"
GGGGS

SEQ ID NO: 482 - protein, 4 aa, unidentified
  REGION 1..4: note = source = /note="Description of Unknown: KDEL retention sequence"
KDEL

SEQ ID NO: 483 - protein, 5 aa, synthetic construct
  REGION 1..5: note = source = /note="Description of Artificial Sequence: Synthetic peptide"
EAAAK

SEQ ID NO: 484 - protein, 7 aa, synthetic construct
  REGION 1..7: note = source = /note="Description of Artificial Sequence: Synthetic peptide"
GSGGGGS

SEQ ID NO: 485 - protein, 15 aa, synthetic construct
  REGION 1..15: note = source = /note="Description of Artificial Sequence: Synthetic peptide"
GGGGSGGGGSGGGGS

SEQ ID NO: 486 - protein, 18 aa, synthetic construct
  REGION 1..18: note = source = /note="Description of Artificial Sequence: Synthetic peptide"
GGSGGSGGSGGSGGSGGS

SEQ ID NO: 487 - protein, 336 aa, unidentified
  REGION 1..336: note = source = /note="Description of Unknown: ADAR1DD-WT sequence"
SLGTGNRCVKGDSLSLKGETVNDCHAEIISRRGFIRFLYSELMKYNSQTAKDSIFEPAKGGEKLQIKKTVSFHLYISTAPCGDGALFDKSCSDRAMESTESRHYPVFENPKQGKLRTKVENGEGTIPVESSDIVPTWDGIRLGERLRTMSCSDKILRWNVLGLQGALLTHFLQPIYLKSVTLGYLFSQGHLTRAICCRVTRDGSAFEDGLRHPFIVNHPKVGRVSIYDSKRQSGKTKETSVNWCLADGYDLEILDGTRGTVDGPRNELSRVSKKNIFLLFKKLCSFRYRRDLLRLSYGEAKKAARDYETAKNYFKKGLKDMGYGNWISKPQEEKNF

SEQ ID NO: 488 - protein, 336 aa, synthetic construct
  REGION 1..336: note = source = /note="Description of Artificial Sequence: Synthetic polypeptide"
SLGTGNRCVKGDSLSLKGETVNDCHAEIISRRGFIRFLYSELMKYNSQTAKDSIFEPAKGGEKLQIKKTVSFHLYISTAPCGDGALFDKSCSDRAMESTESRHYPVFENPKQGKLRTKVENGQGTIPVESSDIVPTWDGIRLGERLRTMSCSDKILRWNVLGLQGALLTHFLQPIYLKSVTLGYLFSQGHLTRAICCRVTRDGSAFEDGLRHPFIVNHPKVGRVSIYDSKRQSGKTKETSVNWCLADGYDLEILDGTRGTVDGPRNELSRVSKKNIFLLFKKLCSFRYRRDLLRLSYGEAKKAARDYETAKNYFKKGLKDMGYGNWISKPQEEKNF

SEQ ID NO: 489 - protein, 385 aa, unidentified
  REGION 1..385: note = source = /note="Description of Unknown: ADAR2DD-WT sequence"
QLHLPQVLADAVSRLVLGKFGDLTDNFSSPHARRKVLAGVVMTTGTDVKDAKVISVSTGTKCINGEYMSDRGLALNDCHAEIISRRSLLRFLYTQLELYLNNKDDQKRSIFQKSERGGFRLKENVQFHLYISTSPCGDARIFSPHEPILEEPADRHPNRKARGQLRTKIESGEGTIPVRSNASIQTWDGVLQGERLLTMSCSDKIARWNVVGIQGSLLSIFVEPIYFSSIILGSLYHGDHLSRAMYQRISNIEDLPPLYTLNKPLLSGISNAEARQPGKAPNFSVNWTVGDSAIEVINATTGKDELGRASRLCKHALYCRWMRVHGKVPSHLLRSKITKPNVYHESKLAAKEYQAAKARLFTAFIKAGLGAWVEKPTEQDQFSLT

SEQ ID NO: 490 - protein, 385 aa, synthetic construct
  REGION 1..385: note = source = /note="Description of Artificial Sequence: Synthetic polypeptide"
QLHLPQVLADAVSRLVLGKFGDLTDNFSSPHARRKVLAGVVMTTGTDVKDAKVISVSTGTKCINGEYMSDRGLALNDCHAEIISRRSLLRFLYTQLELYLNNKDDQKRSIFQKSERGGFRLKENVQFHLYISTSPCGDARIFSPHEPILEEPADRHPNRKARGQLRTKIESGQGTIPVRSNASIQTWDGVLQGERLLTMSCSDKIARWNVVGIQGSLLSIFVEPIYFSSIILGSLYHGDHLSRAMYQRISNIEDLPPLYTLNKPLLSGISNAEARQPGKAPNFSVNWTVGDSAIEVINATTGKDELGRASRLCKHALYCRWMRVHGKVPSHLLRSKITKPNVYHESKLAAKEYQAAKARLFTAFIKAGLGAWVEKPTEQDQFSLT

SEQ ID NO: 491 - protein, 198 aa, synthetic construct [sequence omitted]

SEQ ID NO: 492 - protein, 208 aa, synthetic construct
  REGION 1..208: note = source = /note="Description of Artificial Sequence: Synthetic polypeptide"
MTDAEYVRIHEKLDIYTFKKQFFNNKKSVSHRCYVLFELKRRGERRACFWGYAVNKPQSGTERGIHAEIFSIRKVEEYLRDNPGQFTINWYSSWSPCADCAEKILEWYNQELRGNGHTLKIWACKLYYEKNARNQIGLWNLRDNGVGLNVMVSEHYQCCRKIFIQSSHNQLNENRWLEKTLKRAEKRRSELSIMIQVKILHTTKSPAV

SEQ ID NO: 493 - protein, 229 aa, synthetic construct [sequence omitted]